European Patent Application EP 4 715 045 A1, published March 25, 2026. Title: 변이체 폴리펩티드 및 이를 이용한 L-발린 생산 방법. Applicant: 씨제이제일제당 주식회사. Application KR. The sequence listing filed with the application follows.

SEQUENCE LISTING (29 sequences)

SEQ ID NO: 1 - protein, 172 aa, Corynebacterium glutamicum
MANSDVTRHILSVLVQDVDGIISRVSGMFTRRAFNLVSLVSAKTETLGINRITVVVDADELNIEQITKQLNKLIPVLKVVRLDEETTIARAIMLVKVSADSTNRPQIVDAANIFRARVVDVAPDSVVIESTGTPGKLRALLDVMEPFGIRELIQSGQIALNRGPKTMAPAKI

SEQ ID NO: 2 - DNA, 519 bp, Corynebacterium glutamicum
  source 1..519: mol_type = other DNA
atggctaattctgacgtcacccgccacatcctgtccgtactcgttcaggacgtagacggaatcatttcccgcgtatcaggtatgttcacccgacgcgcattcaacctcgtgtccctcgtgtctgcaaagaccgaaacactcggcatcaaccgcatcacggttgttgtcgacgccgacgagctcaacattgagcagatcaccaagcagctcaacaagctgatccccgtgctcaaagtcgtgcgacttgatgaagagaccaccatcgcccgcgcaatcatgctggttaaggtctctgcggatagcaccaaccgtccgcagatcgtcgacgccgcgaacatcttccgcgcccgagtcgtcgacgtggctccagactctgtggttattgaatccacaggcaccccaggcaagctccgcgcactgcttgatgtgatggaaccattcggaatccgcgaactgatccaatccggacagattgcactcaaccgcggtccgaagaccatggctccggccaagatctaa

SEQ ID NO: 3 - protein, 172 aa, synthetic construct
MANSDVTRHILSVLVQDVDGIISRVSGMFTRRAFNLVSLVSAKTETLGINRITVVVDADELNIEQITKQLNKLIPVLKVVRLDEETTIARAIMLVKVSADSTNRPQIVDAANIFRARVVDVAPDSVVIESTGTPGKLRALLDVMEPFGIRELIRSGQIALNRGPKTMAPAKI

SEQ ID NO: 4 - DNA, 519 bp, synthetic construct
  source 1..519: mol_type = other DNA
atggctaattctgacgtcacccgccacatcctgtccgtactcgttcaggacgtagacggaatcatttcccgcgtatcaggtatgttcacccgacgcgcattcaacctcgtgtccctcgtgtctgcaaagaccgaaacactcggcatcaaccgcatcacggttgttgtcgacgccgacgagctcaacattgagcagatcaccaagcagctcaacaagctgatccccgtgctcaaagtcgtgcgacttgatgaagagaccaccatcgcccgcgcaatcatgctggttaaggtctctgcggatagcaccaaccgtccgcagatcgtcgacgccgcgaacatcttccgcgcccgagtcgtcgacgtggctccagactctgtggttattgaatccacaggcaccccaggcaagctccgcgcactgcttgatgtgatggaaccattcggaatccgcgaactgatccgatccggacagattgcactcaaccgcggtccgaagaccatggctccggccaagatctaa

SEQ ID NO: 5 - protein, 172 aa, synthetic construct
MANSDVTRHILSVLVQDVDGIISRVSGMFTRRAFNLVSLVSVKTETLGINRITVVVDADELNIEQITKQLNKLIPVLKVVRLDEETTIARAIMLVKVSADSTNRPQIVDAANIFRARVVDVAPDSVVIESTGTPGKLRALLDVMEPFGIRELIRSGQIALNRGPKTMAPAKI

SEQ ID NO: 6 - DNA, 519 bp, synthetic construct
  source 1..519: mol_type = other DNA
atggctaattctgacgtcacccgccacatcctgtccgtactcgttcaggacgtagacggaatcatttcccgcgtatcaggtatgttcacccgacgcgcattcaacctcgtgtccctcgtgtctgtaaagaccgaaacactcggcatcaaccgcatcacggttgttgtcgacgccgacgagctcaacattgagcagatcaccaagcagctcaacaagctgatccccgtgctcaaagtcgtgcgacttgatgaagagaccaccatcgcccgcgcaatcatgctggttaaggtctctgcggatagcaccaaccgtccgcagatcgtcgacgccgcgaacatcttccgcgcccgagtcgtcgacgtggctccagactctgtggttattgaatccacaggcaccccaggcaagctccgcgcactgcttgatgtgatggaaccattcggaatccgcgaactgatccgatccggacagattgcactcaaccgcggtccgaagaccatggctccggccaagatctaa

SEQ ID NO: 7 - protein, 172 aa, synthetic construct
MANSDVTRHILSVLVQDVDGIISRVSGMFTRRAFNLVSLVSAKTETLGINRITVVVDADELNIEQITKQLNKLIPVLKVVRLDEETTIARAIMLVKVSADSTNRPQIVDAANIFRARVVDVAPDSVVIESTGTPGKLRALLDVMEPFGIRELIHSGQIALNRGPKTMAPAKI

SEQ ID NO: 8 - protein, 172 aa, synthetic construct
MANSDVTRHILSVLVQDVDGIISRVSGMFTRRAFNLVSLVSAKTETLGINRITVVVDADELNIEQITKQLNKLIPVLKVVRLDEETTIARAIMLVKVSADSTNRPQIVDAANIFRARVVDVAPDSVVIESTGTPGKLRALLDVMEPFGIRELIESGQIALNRGPKTMAPAKI

SEQ ID NO: 9 - protein, 172 aa, synthetic construct
MANSDVTRHILSVLVQDVDGIISRVSGMFTRRAFNLVSLVSVKTETLGINRITVVVDADELNIEQITKQLNKLIPVLKVVRLDEETTIARAIMLVKVSADSTNRPQIVDAANIFRARVVDVAPDSVVIESTGTPGKLRALLDVMEPFGIRELIHSGQIALNRGPKTMAPAKI

SEQ ID NO: 10 - protein, 172 aa, synthetic construct
MANSDVTRHILSVLVQDVDGIISRVSGMFTRRAFNLVSLVSVKTETLGINRITVVVDADELNIEQITKQLNKLIPVLKVVRLDEETTIARAIMLVKVSADSTNRPQIVDAANIFRARVVDVAPDSVVIESTGTPGKLRALLDVMEPFGIRELIESGQIALNRGPKTMAPAKI

SEQ ID NO: 11 - DNA, 25 bp, synthetic construct
  source 1..25: mol_type = other DNA
cccgggatggctaattctgacgtca

SEQ ID NO: 12 - DNA, 25 bp, synthetic construct
  source 1..25: mol_type = other DNA
cccgggtgtctggagccaggagcat

SEQ ID NO: 13 - DNA, 41 bp, synthetic construct
  source 1..41: mol_type = other DNA
cggggatcccccgggaggacggtactcaaatactaaacttc

SEQ ID NO: 14 - DNA, 38 bp, synthetic construct
  source 1..38: mol_type = other DNA
tgccgagtgtttcggtctttacagacacgagggacacg

SEQ ID NO: 15 - DNA, 31 bp, synthetic construct
  source 1..31: mol_type = other DNA
tgtctgtaaagaccgaaacactcggcatcaa

SEQ ID NO: 16 - DNA, 41 bp, synthetic construct
  source 1..41: mol_type = other DNA
cggggatcccccggggacaactacattattattataccaca

SEQ ID NO: 17 - DNA, 18 bp, synthetic construct
  source 1..18: mol_type = other DNA
ccgcgtcaccaaagcgga

SEQ ID NO: 18 - DNA, 20 bp, synthetic construct
  source 1..20: mol_type = other DNA
ttagatcttggccggagcca

SEQ ID NO: 19 - DNA, 23 bp, synthetic construct
  source 1..23: mol_type = other DNA
cgaactgatccactccggacaga

SEQ ID NO: 20 - DNA, 23 bp, synthetic construct
  source 1..23: mol_type = other DNA
tctgtccggagtggatcagttcg

SEQ ID NO: 21 - DNA, 23 bp, synthetic construct
  source 1..23: mol_type = other DNA
cgaactgatcgagtccggacaga

SEQ ID NO: 22 - DNA, 23 bp, synthetic construct
  source 1..23: mol_type = other DNA
tctgtccggactcgatcagttcg

SEQ ID NO: 23 - protein, 10 aa, synthetic construct
  source 1..10: note = X =R or H or E
EPFGIRELIX

SEQ ID NO: 24 - protein, 21 aa, synthetic construct
  source 1..21: note = X =R or H or E
PGKLRALLDVLEPFGIRELIX

SEQ ID NO: 25 - protein, 107 aa, synthetic construct
  source 1..107: note = X =R or H or E
GINRITVVVDADELNIEQITKQLNKLIPVLKVVRLDEETTIARAIMLVKVSADSTNRPQIVDAANIFRARVVDVAPDSVVIESTGTPGKLRALLDVMEPFGIRELIX

SEQ ID NO: 26 - protein, 8 aa, synthetic construct
NLVSLVSV

SEQ ID NO: 27 - protein, 32 aa, synthetic construct
LSVLVQDVDGIISRVSGMFTRRAFNLVSLVSV

SEQ ID NO: 28 - protein, 42 aa, synthetic construct
MANSDVTRHILSVLVQDVDGIISRVSGMFTRRAFNLVSLVSV

SEQ ID NO: 29 - DNA, 5802 bp, synthetic construct
  source 1..5802: mol_type = other DNA
gttcgcttgctgtccataaaaccgcccagtctagctatcgccatgtaagcccactgcaagctacctgctttctctttgcgcttgcgttttcccttgtccagatagcccagtagctgacattcatccggggtcagcaccgtttctgcggactggctttctacgtgttccgcttcctttagcagcccttgcgccctgagtgcttgcggcagcgtgaagctagcttttatcgccattcgccattcaggctgcgcaactgttgggaagggcgatcggtgcgggcctcttcgctattacgccagctggcgaaagggggatgtgctgcaaggcgattaagttgggtaacgccagggttttcccagtcacgacgttgtaaaacgacggccagtgaattcgagctcggtacccggggatcctctagagtcgacctgcaggcatgcaagcttggcgtaatcatggtcatagctgtttcctgtgtgaaattgttatccgctcacaattccacacaacatacgagccggaagcataaagtgtaaagcctggggtgcctaatgagtgagctaactcacattaattgcgttgcgctcactgcccgctttccagtcgggaaacctgtcgtgccagctgcattaatgaatcggccaacgcgcggggagaggcggtttgcgtattgggcgctcttccgcttcctcgctcactgactcgctgcgctcggtcgttcggctgcggcgagcggtatcagctcactcaaaggcggtaatacggttatccacagaatcaggggataacgcaggaaagaacatgtgagcaaaaggccagcaaaaggccaggaaccgtaaaaaggccgcgttgctggcgtttttccataggctccgcccccctgacgagcatcacaaaaatcgacgctcaagtcagaggtggcgaaacccgacaggactataaagataccaggcgtttccccctggaagctccctcgtgcgctctcctgttccgaccctgccgcttaccggatacctgtccgcctttctcccttcgggaagcgtggcgctttctcaatgctcacgctgtaggtatctcagttcggtgtaggtcgttcgctccaagctgggctgtgtgcacgaaccccccgttcagcccgaccgctgcgccttatccggtaactatcgtcttgagtccaacccggtaagacacgacttatcgccactggcagcagccactggtaacaggattagcagagcgaggtatgtaggcggtgctacagagttcttgaagtggtggcctaactacggctacactagaaggacagtatttggtatctgcgctctgctgaagccagttaccttcggaaaaagagttggtagctcttgatccggcaaacaaaccaccgctggtagcggtggtttttttgtttgcaagcagcagattacgcgcagaaaaaaaggatctcaagaagatcctttgatcttttctacggggtctgacgctcagtggaacgaaaactcacgttaagggattttggtcatgagattatcaaaaaggatcttcacctagatccttttggggtgggcgaagaactccagcatgagatccccgcgctggaggatcatccagccctgatagaaacagaagccactggagcacctcaaaaacaccatcatacactaaatcagtaagttggcagcatcacccgacgcactttgcgccgaataaatacctgtgacggaagatcacttcgcagaataaataaatcctggtgtccctgttgataccgggaagccctgggccaacttttggcgaaaatgagacgttgatcggcacgtaagaggttccaactttcaccataatgaaataagatcactaccgggcgtattttttgagttatcgagattttcaggagctgatagaaacagaagccactggagcacctcaaaaacaccatcatacactaaatcagtaagttggcagcatcacccgacgcactttgcgccgaataaatacctgtgacggaagatcacttcgcagaataaataaatcctggtgtccctgttgataccgggaagccctgggccaacttttggcgaaaatgagacgttgatcggcacgtaagaggttccaactttcaccataatgaaataagatcactaccgggcgtattttttgagttatcgagattttcaggagctctttggcatcgtctctcgcctgtcccctcagttcagtaatttcctgcatttgcctgtttccagtcggtagatattccacaaaacagcagggaagcagcgcttttccgctgcataaccctgcttcggggtcattatagcgattttttcggtatatccatcctttttcgcacgatatacaggattttgccaaagggttcgtgtagactttccttggtgtatccaacggcgtcagccgggcaggataggtgaagtaggcccacccgcgagcgggtgttccttcttcactgtcccttattcgcacctggcggtgctcaacgggaatcctgctctgcgaggctggccggctaccgccggcgtaacagatgagggcaagcggatggctgatgaaaccaagccaaccaggaagggcagcccacctatcaaggtgtactgccttccagacgaacgaagagcgattgaggaaaaggcggcggcggccggcatgagcctgtcggcctacctgctggccgtcggccagggctacaaaatcacgggcgtcgtggactatgagcacgtccgcgagggcgtcccggaaaacgattccgaagcccaacctttcatagaaggcggcggtggaatcgaaatctcgtgatggcaggttgggcgtcgcttggtcggtcatttcgaaaaaggttaggaatacggttagccatttgcctgcttttatatagttcatatgggattcacctttatgttgataagaaataaaagaaaatgccaataggatatcggcattttcttttgcgtttttatttgttaactgttaattgtccttgttcaaggatgctgtctttgacaacagatgttttcttgcctttgatgttcagcaggaagctcggcgcaaacgttgattgtttgtctgcgtagaatcctctgtttgtcatatagcttgtaatcacgacattgtttcctttcgcttgaggtacagcgaagtgtgagtaagtaaaggttacatcgttaggcggatcaagatccatttttaacacaaggccagttttgttcagcggcttgtatgggccagttaaagaattagaaacataaccaagcatgtaaatatcgttagacgtaatgccgtcaatcgtcatttttgatccgcgggagtcagtgaacaggtaccatttgccgttcattttaaagacgttcgcgcgttcaatttcatctgttactgtgttagatgcaatcagcggtttcatcacttttttcagtgtgtaatcatcgtttagctcaatcataccgagagcgccgtttgctaactcagccgtgcgttttttatcgctttgcagaagtttttgactttcttgacggaagaatgatgtgcttttgccatagtatgctttgttaaataaagattcttcgccttggtagccatcttcagttccagtgtttgcttcaaatactaagtatttgtggcctttatcttctacgtagtgaggatctctcagcgtatggttgtcgcctgagctgtagttgccttcatcgatgaactgctgtacattttgatacgtttttccgtcaccgtcaaagattgatttataatcctctacaccgttgatgttcaaagagctgtctgatgctgatacgttaacttgtgcagttgtcagtgtttgtttgccgtaatgtttaccggagaaatcagtgtagaataaacggatttttccgtcagatgtaaatgtggctgaacctgaccattcttgtgtttggtcttttaggatagaatcatttgcatcgaatttgtcgctgtctttaaagacgcggccagcgtttttccagctgtcaatagaagtttcgccgactttttgatagaacatgtaaatcgatgtgtcatccgcatttttaggatctccggctaatgcaaagacgatgtggtagccgtgatagtttgcgacagtgccgtcagcgttttgtaatggccagctgtcccaaacgtccaggccttttgcagaagagatatttttaattgtggacgaatcaaattcagaaacttgatatttttcatttttttgctgttcagggatttgcagcatatcatggcgtgtaatatgggaaatgccgtatgtttccttatatggcttttggttcgtttctttcgcaaacgcttgagttgcgcctcctgccagcagtgcggtagtaaaggttaatactgttgcttgttttgcaaactttttgatgttcatcgttcatgtctccttttttatgtactgtgttagcggtctgcttcttccagccctcctgtttgaagatggcaagttagttacgcacaataaaaaaagacctaaaatatgtaaggggtgacgccaaagtatacactttgccctttacacattttaggtcttgcctgctttatcagtaacaaacccgcgcgatttacttttcgacctcattctattagactctcgtttggattgcaactggtctattttcctcttttgtttgatagaaaatcataaaaggatttgcagactacgggcctaaagaactaaaaaatctatctgtttcttttcattctctgtattttttatagtttctgttgcatgggcataaagttgcctttttaatcacaattcagaaaatatcataatatctcatttcactaaataatagtgaacggcaggtatatgtgatgggttaaaaaggatcaccccagagtcccgctcagaagaactcgtcaagaaggcgatagaaggcgatgcgctgcgaatcgggagcggcgataccgtaaagcacgaggaagcggtcagcccattcgccgccaagctcttcagcaatatcacgggtagccaacgctatgtcctgatagcggtccgccacacccagccggccacagtcgatgaatccagaaaagcggccattttccaccatgatattcggcaagcaggcatcgccatgggtcacgacgagatcctcgccgtcgggcatccgcgccttgagcctggcgaacagttcggctggcgcgagcccctgatgctcttcgtccagatcatcctgatcgacaagaccggcttccatccgagtacgtgctcgctcgatgcgatgtttcgcttggtggtcgaatgggcaggtagccggatcaagcgtatgcagccgccgcattgcatcagccatgatggatactttctcggcaggagcaaggtgagatgacaggagatcctgccccggcacttcgcccaatagcagccagtcccttcccgcttcagtgacaacgtcgagacagctgcgcaaggaacgcccgtcgtggccagccacgatagccgcgctgcctcgtcttggagttcattcagggcaccggacaggtcggtcttgacaaaaagaaccgggcgcccctgcgctgacagccggaacacggcggcatcagagcagccgattgtctgttgtgcccagtcatagccgaatagcctctccacccaagcggccggagaacctgcgtgcaatccatcttgttcaatcatgcgaaacgatcctcatcctgtctcttgatcagatcttgatcccctgcgccatcagatccttggcggcaagaaagccatccagtttactttgcagggcttcccaaccttaccagagggcgccccagctggcaattccg